European Patent Specification EP 4 466 381 B1, published August 5, 2026. Title: Ori-C MEDIATED EXTRACHROMOSOMAL DNA AMPLIFICATION AND SEQUENCING FOR DIAGNOSING, SCREENING AND TREATING DISEASE. Applicant: The Jackson Laboratory. Application US. The sequence listing filed with the application follows.

SEQUENCE LISTING (10 sequences)

SEQ ID NO: 1 - DNA, 38 bp, synthetic construct
  source 1..38: mol_type = other DNA
ctgtctcttatacacatctctgctctgatgccgcatag

SEQ ID NO: 2 - DNA, 38 bp, synthetic construct
  source 1..38: mol_type = other DNA
ctgtctcttatacacatctgtgtcggggctggcttaac

SEQ ID NO: 3 - DNA, 46 bp, synthetic construct
  source 1..46: mol_type = other DNA
ctgtctcttatacacatctgcccgggcctgctctgatgccgcatag

SEQ ID NO: 4 - DNA, 46 bp, synthetic construct
  source 1..46: mol_type = other DNA
ctgtctcttatacacatctgcccgggcgtgtcggggctggcttaac

SEQ ID NO: 5 - DNA, 46 bp, synthetic construct
  source 1..46: mol_type = other DNA
ctgtctcttatacacatctgtttaaacctgctctgatgccgcatag

SEQ ID NO: 6 - DNA, 46 bp, synthetic construct
  source 1..46: mol_type = other DNA
ctgtctcttatacacatctgtttaaacgtgtcggggctggcttaac

SEQ ID NO: 7 - DNA, 472 bp, synthetic construct
  source 1..472: mol_type = other DNA
ctgtctcttatacacatctgaagatccggcagaagaatggagtatgttgtaactaaagataacttcgtataatgtatgctatacgaagttatacagatcgtgcgatctactgtggataactctgtcaggaagcttggatcaaccggtagttatccaaagaacaactgttgttcagtttttgagttgtgtataacccctcattctgatcccagcttatacggtccaggatcaccgatcattcacagttaatgatcctttccaggttgttgatcttaaaagccggatccttgttatccacagggcagtgcgatcctaataagagatcacaatagaacagatctctaaataaatagatcttctttttaatacccaggatccatctatgtcgggtgcggagaaagaggtaatgaaatggctttagttacaacatactcaggtctttctcaagccgacagatgtgtataagagacag

SEQ ID NO: 8 - DNA, 4530 bp, unidentified
  source 1..4530: mol_type = genomic DNA
cttgtacttcgttcagttacgtattgctgtacttcgttcagttacgtgtgctgggcagatgtgtataagagacaggcttggctggcttggctggctgggtggcttgcctggcttggctggcttggctggatggctggcttgactggcttggctcgctggctgccctggctggctggatggctggctggctggctggcttggctggctggctggctggctggcttggctggctggctggcttggctggcttggctggctggctggcttggctggctggctggcttggctggctggctgggctggctggctggctggctttggctgccctggcttggctggctctggctggctgactggctggctggattggctagcttggctggccggctggcttggcaggctggatggctctggctggcttggctggcaggctggtttctctcttgggtgtcttggctggcttggctggcttggctggctggctctctggctctgtggctggctggctggctggctggcttggctggctggcttggctggcttggctggcttggctggctggcttgcttggctggctggcttggctggctctggctggcttggctggctggctggcttggctggcttggctggctggctggcttggctggctctggctggcttggctggctggctggctggctggctggctggctggctggctggctggctggctgctggctggcttggctggctggctggctggctggcttggctggctggctggctggctggctggctggctggctggctggctggctggctggctggctggctggctggctggctggctggctggctggctggctggctggctggctgggctggctggctggctggctggagagctggctggagagagagagctggagagagagagagcttggagagagagagagagctggctggctggagagctggagagagagagagagagagagagaggctggcttgagagagagagagagagagagagagagagagagagagagagagagagagagagagctggagagagagagagagagagagctggcttggctggctggctggctggagagagagagagagagctggcttggctggctggctggagagagagagagagagagagagagagagagagctggctggctggagagagagctggctggagagagagagagagagagagagagagagagagagagagagagagagagagagagagagagagagagagagagagagagagagagagagagagagagagagcttggagagaggagagagagaggctggctggagagagagagagagagagagagagagaggctgagagagagagagctggagagagagagagagagagcagagagagagagagagagaggagagagagagagagagagcttggagagagagaggagagagagagagagagagagagagagagagagagagagagagagagagagagagagagagagagagagagagagagagagagagctggagagagagagagagagagagaggagagagagagagagagagagagagctctggagagagagagagagagagagctgagagagaggaggctggagagagagagagagagagagagagagagagagagagagagagagagagagagagagagagagagagagagagagagagagactgagagagagagagagagagagagagagagagagagagagagagagagagagagagagagagagagagagagagagagagagagagagagagctgagctggagagagagagagagagagagagagagagagagagagagagagagagagagagagagagagagagctgagagagagagagagagagagagagagagagagagagagagagagagagagagagagagagagagagagagagagagagagagagagagagagagagagagagagagagagagagagagagagagagagagagagagagagagagagagaggctctctctgagagaggctggagagagagagagcttgagagagctggctggctggagagagagagagagagagagagagagagagagagagagagagctggagagagagagagagagagagagagagagagagagctggagagagagctctgctctctctctggcttggctggctggctggctgagagagagagctggctggcttggctggctggctggctggctctgagagagctgagctggagagagagagagctctggctggctggcttggctggctctggctggctggctggctggctgagctggctggctggctggagagagagagctggctctggctggagagagactggctggctggctggctgagctggctctggctggctggctggctggctctggctggctctctgagagagagagagctggctggctggagagctgagctctctggctggctggctggctgctggctggctgctggctgagagagctgagctggctggctggctctggctgaggctgagaggcttggctggctggctggagagaggagctggctggctggctggctgggcttggctggctggctggctggctggctggctgagctggagctgagagagaggctgagctgaggctgctggctggcttggctggctgctctgctgctggagctggctggctggctggctggctggctctggctggctggctggctctgctggctctggctgctggctggctggctggctggctggctggctggctggctctggctggctggcttggctggctggctatgcttggctggctggctggctggctggcttggctgagagctggctggctggctggctggctggctggctggctctgctggctggctctgctggctgagctggcttggctgagctctctgctggctggctggagcttggctggagctggcttggctgagagctggctggctggctggctggcttggctggctggctggcttggctggctggctggctggctggctggctggctggctggctggctggcttggctggctggctggctggctggcttggctggctggctggctggctgagctggctggctggctctggctggagctggctggctggctggctggctggctggctggctggctggctggctgatcttggctgggctggctggctggctggctggctggctggctgctgagcttggctggctggcttggctggctgctggctggcttggctggctggctgagctggatggctggctggctgagctggctggcttggctggctggctggctggctggcttggctggctggctgctggagctggctggctggctggctggctggctggctggctggctggctggctggctggctggcttggctggctggctggctggctggctggagagagagagagctggctggctggctggcttggctggctggctggctggctggctggctggctggctggaggctggctggagaggcttggctggctggctggctggctggctggctggctgagcttggctggcttggctggagagagagagagaggctggctggctgagagctggctggctggcttggctggctggctggctggctggctggagagctggagctggctggctggctggctggctggctgagagcttggctggctggctggctggctggctggctggagagagagagagagctggctggagagctggctggctggagctggcttggctggcttggctggctggagagagactggctggctggagagctgagagctggctggagagagagagaggctggctggctggctggctggcagctggcttggctggctggctggctggctggctggctggctggctggcttggctggcttggctggagaggctggctggctggctggctggctggagagctggctgagctggctggctggctggctggctggctggctggctggctgagctggcttggctggctggctggctggctggcttggctggctggctggctggctggctggctggctggctggctgggagagagagagagagagagagagagagagagagagctggctggctggctgagagagagaggagctggaggctggctggctggctgagctggctggcttggagctggctggctggagagctggctggcactggctggagagagagagaggctggctggctgggagagagagagagagagagagagagagagctgacacactggctggctggcttggctggcttggctggctgtgtggctggctggctggagagagagagagagctggagagctggctggctgagaggctggcatgagctggctgagctggcagagaggtggctggcttggctggcttgagagagagagagagtggctggcctgactggctgagagagagagagctgtctcttatacacatctgcccagcaagcaatacttgcaat

SEQ ID NO: 9 - DNA, 3961 bp, unidentified
  source 1..3961: mol_type = genomic DNA
acttgtacttcttgtacttcgttcagttacgtattgctgggcagatgtgtataagagacaggcttggctggcttggctggctgggtggcttgcctggcttggctggcttggctggatggctggcttgactggcttggctcgctggctgctggctgctggcttggctggctggctggctgctggcttggctggctggctggcttggctggctggctggctggcttggctggctggctggcttggctggctggctggctggctggcttggctggctggctggctggctggctggctggcttggctggctggctggctggcttggatggctggctggcttggctggcttggctggcttggctggcttggtggctgccagcttggcaggccttggcttggcttgctgccagcttgctggcttggctggctggagctggctggctggcttgggctggctggcttggctggctggctggctggctggcttggctggcaggctggcttggctggctcttgggtgggctggctgggctggcttggctggctggctggctggctggctggctgtggggctggctggcttggctggctggctggctggcttggctgggctggctggctggcttggctggctggcttggctggcttggctggctggctggctggtggctggctggcttggctggctggctgggctggctggcttggctggctggctggctggcttggctggctggctggcttggctggctggctggctggctggctggctggctggctggagctggctggctggctggctggcttggctggggctggctggctggctggctggctggctggctggctggctggctggcttggctggcttggctggctggctgggctggctgggctggctggctggctggctggctggctgccagctggctggctggctggctggctggctggctggctggctggctgggctgctggcttggctggctggctggctggctggctggctggcttggctggccatggctggctggctggctgggctggctggcttggctggcttggctggctggctggctggctggctggctggctggctggccaagctggctggctggctgggctggctggctggctgggctgcagctggctggctggctggctggctggagagagctgcagctggctggctggcagcctgcttggctggctggctggcttggccagccaggctggctggagaagccagcttggctggctggccagctgggatggctagctggcttggagccagctggagaggagcctggctggctggctggcttggctggctggctgcttggctggctggctggctggagcctggctggctgcttgagctggctggctggctggctggctggctggctggctggctggctgagctggcagctggctggctggctggctggccagcagcagccaggcagctggctggctggctggctggcagcttggctggccagcttggctgagagagctggctggctggctggcagccagcctggcttggctggctggctggccaggctgctggctggcagctggctggcttggctggctgggctggctggcttggctggcttggctggctggctggctggctggctggcaaggctggcagcctggctggccagctggctggcttggctggcctggcagctggctggccagctggctggcagccagctggcccagcctggctggctggcagccagccagctggccagctgctggctggcaggctgctgctggctggctggctggcctggctggctggcctggcttggccttggctggctggctggctggctggctggctggctgctgcaagccagctggcctggctgcctggcctggcttggctggctggctggcttggctggctggctggctggctggctggcttctggccaggctggctggcttggctggctggcctggccagccagctgctggcaaggctggctggcagccagctggctggccaggctggccagcagctggctggctggctggctggctggctgagcctggctggctggctggctggccagctggctgccaagcctggctggaggcctggctggcttggctggcttggcttggctggctggccagccaggccagccagctggctggcctggagcctgcctggagttaatgagctggcttggctgccagctggcctggctggcttggctggcttggctggctggctggctggctggctgaggctggctggctggctgccagctggctggctggctggccaggctgcagctgagctggcaggcttctggctggctgcttggctagctggctggctgtctctggctctggctggctggctggctggccagcctggcagcctggcagccagctggcttggctggctggctctggctggctggctggctgccagctggctggcttcagctggctggagcagatctctctccagccagccagcagcagagctggccaagccagctggctggcagagccagccagcaagcatcagccagccagagccagagagcagagcctgctgcctgagagagagagagccagagatcagagagctgagagagagagagagagagagagagagagagagctcagccagagagaaagccagctgccagccacagagagagagctgccagagagagagagccagagagagagagagagagagaaagagagagagctctggctggcttggcagagagagccagaggccagccagagctggctctgccagccagagagagagagagctccagagagctggctgagcagagcagctggagagagagagagagcagccaggctgagcagctggcaggctggcagcctgccagctctgagcagagctcagagctgagctctctctctggctgagagagctggagagagagagagagagagaccagccagagagagccagagccagccagagagctggcacagcagagagagcttgagagacagagagagagagagacagagagagagagagagagccagagagagagagagagccagacagagagagagagagagagagagagagagagcctgagagagagagagagaggctgagagagccagagagagagagagagagctgagagagagagagagagcctctctctctctgccagctgagagagaggctctcagagccagctggctcagcagagagactctctctgagagagacagagagctgagctctgagctggctgagagagagagagagagagagagagagagagagagagagagagctctctcagagagagagagagagagagagagctctctgagcttgagagagagagagagagagccagagagacagccagctggagagagagagagagagacaggacagcacacactgagctcccagagagagagagagagagagagagagagagagagagagagagagagagagagtgagagagagagagagagctgagagagagagagcagcttggctgagctgagagagagagctgagagagagagagcctgagagcacagaggctggctgagagagagagagagagagagagagagagagagagcttggagagagagagagagagagagagagagagacagagcagccaagagcagctggctctgagagagctgagctgagctggctctggctggctgctggctggagagagagagagagagagagagagagagagagagccagagagagagagagagcagagagagagagagctgacagagagagagacagagagccttggctgagagagagagagagagagagagagagagagagagagaagagagagagagagagagagagagagagctgtctcttatcttatacacatactgcccagcaatctgcccagcaatacgtaagaga

SEQ ID NO: 10 - DNA, 2116 bp, unidentified
  source 1..2116: mol_type = genomic DNA
acaaacatacttgtacttcgttcagttacgtattgctgggcgtgtacttcgttcagttacgtattgctgggcagatgtgtataagagacagccatctagccatccagccagtcaggccagccacccagccaagccagccaagccagccaagccagccacccgccaagccagccagccagccatgccagccagccagccagccagccagttacaagcccagtattgcctgcttcgttcagttacgtattgctgggcagatgtgtataagagacagccatctagccatccagccagtcaggccagccacccagccaagccagccaagccagccaagccagccacccagccaagccagccagccagccagccagccaagccagccagccagccagccaagccacccagccagccagccagccaagccacacagccagccagccagccaagccagccagccagccagccagccagccagccagccagccagccagccagccagccagcccagccagccagccagccagccagccagccagccagccagccagccagccagccagccagccagccagccagccagccagccagccagccagccagccagccagccagccagccagcccagccagccagccagccagccagccagccagccagccagccagccagccagccagccagccagccagccagccagccagccagccagccagccaagccagccagccagccagccagccagccagccagccagccagccagccagcccagccagccagccagccagccagccagccagccagccagccagccaagccagccaagccagccaagccagccagccagccaagccagccagccagccagccagccatccgagccagccagccagccagccaagcccagccaagcccagccagccagccatcccagccagtcaagccagccaagccagccaagccagccagccagccaagccagccagccagccagccagccagccagccaagccagccaagccagccaagccagccagccagccagccagccaagccagccaagccagccagccagccaagccagccaagccagccatccagccagccagccaagccagccaagccagcccagccagccaagccagccagccaagccagccagcccagccaagccagccagccagccagccagccagccagccagccagccagccaagccagccaagccagcccagccagccagccagccagccagccagccagccagccagccaagccagccagccagccagccagccagccagccagccagccagccaagccagccagccagccaagccagccaagccagccaagccagccagccagccagccagccaagccccagcctcaagccagccagccagccaagccagccagccagccagccagccagccagccagccaagccagccaagccaagctcttatacacagccagccagccagccagccagccaagccagccagcccagccagccagccagccagccagccagccagccaaccagccagccagccagccagccaagccagccagccagccagccagccagccaagccagccagccagccatccagccaagccagccagccagccaagccagcccagccagccaagccagccaagcctgtctcttagccatctgcccagcctagccagcccagccagccagcctttttcagccaagccagccaagtaccaatccctcattctgacccagctgccagccatcatttgccagccagccaaaacctgggcagccaagccagccaagccagcctaatgatccttttccaggttgttgatcaagccagccaagcagccaagccagccagccagcgaaagatcattagcctgtgaagatcagtgatccagataagcctgggatcagccagccatacacaagccaaagccatccaagccagttctttggataactaccggttgagccaagcttccagtcaagacagccatccagttatccagccaagcctttagcacaacatactagccagccaagccagccaagcctgtctcttatacacatctgcccagcaatacgtatgcaatgtgat